European Patent Application EP 4 556 488 A2, published May 21, 2025. Title: NOVEL METHOD FOR PREPARING LONG-ACTING DRUG CONJUGATE THROUGH PREPARATION OF INTERMEDIATE. Applicant: HANMI PHARM. CO., LTD. Application EP. The sequence listing filed with the application follows.

SEQUENCE LISTING (10 sequences)

SEQ ID NO: 1 - protein, 40 aa, synthetic construct
  REGION 1..40: note = GLP-1/GIP/Glucagon Triple Agonist analog 1
  VARIANT 2: note = Xaa = aminoisobutyric acid
YXQGTFTSDYSKYLDEKRAKEFVQWLLDHHPSSGQPPPSC

SEQ ID NO: 2 - protein, 39 aa, synthetic construct
  REGION 1..39: note = GLP-1/GIP/Glucagon Triple Agonist analog 2
  VARIANT 2: note = Xaa = aminoisobutyric acid
YXQGTFTSDYSKYLDEKRAKEFVQWLLDHHCSSGQPPPS

SEQ ID NO: 3 - protein, 40 aa, synthetic construct
  REGION 1..40: note = GLP-1/GIP/Glucagon Triple Agonist analog 3
  VARIANT 2: note = Xaa = aminoisobutyric acid
HXQGTFTSDYSKYLDEKRAKEFVQWLLDHHPSSGQPPPSC

SEQ ID NO: 4 - protein, 30 aa, synthetic construct
  REGION 1..30: note = Glucagon analog 1
  VARIANT 2: note = Xaa = aminoisobutyric acid
YXQGTFTSDYSKYLDEKRAKEFVQWLMNTC

SEQ ID NO: 5 - protein, 29 aa, synthetic construct
  REGION 1..29: note = Glucagon analog 2
  VARIANT 2: note = Xaa = aminoisobutyric acid
YXQGTFTSDYSKYLDECRAKEFVQWLMNT

SEQ ID NO: 6 - protein, 30 aa, synthetic construct
  REGION 1..30: note = Glucagon analog 3
  VARIANT 2: note = Xaa = aminoisobutyric acid
YXQGTFTSDYSKYLDSRRAQDFVQWLMNTC

SEQ ID NO: 7 - protein, 12 aa, Homo sapiens
ESKYGPPCPSCP

SEQ ID NO: 8 - skipped

SEQ ID NO: 9 - protein, 4 aa, synthetic construct
  REGION 1..4: note = Variant of hinge region
PSCP

SEQ ID NO: 10 - protein, 221 aa, Homo sapiens
PSCPAPEFLGGPSVFLFPPKPKDTLMISRTPEVTCVVVDVSQEDPEVQFNWYVDGVEVHNAKTKPREEQFNSTYRVVSVLTVLHQDWLNGKEYKCKVSNKGLPSSIEKTISKAKGQPREPQVYTLPPSQEEMTKNQVSLTCLVKGFYPSDIAVEWESNGQPENNYKTTPPVLDSDGSFFLYSRLTVDKSRWQEGNVFSCSVMHEALHNHYTQKSLSLSLGK